European Patent Application EP 4 617 365 A1, published September 17, 2025. Title: 双链RNA的合成方法及RNA连接酶在双链RNA合成中的应用. Applicant: 凯莱英生命科学技术（天津）有限公司. Application CN. The sequence listing filed with the application follows.

SEQUENCE LISTING (43 sequences)

SEQ ID NO: 1 - protein, 327 aa, Vibrio phage
MSFVKYTSLENSYRQAFVDKCDMLGVRDWVALEKIHGANFSFIVEFDGGYTVTPAKRTSIIGATATGDYDFYGCTSVVEAHKEKVELVANFLWLNEYINLYEPIIIYGELAGKGIQKEVNYGDKDFWAFDIFLPQREEFVDWDTCVAAFTNAEIKYTKELARGTLDELLRIDPLFKSLHTPAEHEGDNVAEGFVVKQLHSEKRLQSGSRAILKVKNEKFKEKKKKEGKTPTKLVLTPEQEKLHAEFSCYLTENRLKNVLSKLGTVNQKQFGMISGLFVKDAKDEFERDELNEVAIDRDDWNAIRRSLTNIANEILRKNWLNILDGNF

SEQ ID NO: 2 - protein, 381 aa, Vibrio phage
MNVQELYKNLMSLADDAEGKFFFADHLSPLGEKFRVFSYHIASYSDWLLPGALEARGIMFQLDDNDEMIRIVSRPMEKFFNLNENPFTMELDLTTTVQLMDKADGSLISTYLSGENFALKSKTSIFSEQAVAANRYIKKPENRDLWEFCDDCTQAGLTVNMEWCAPNNRIVLEYPEAKLVILNIRDNETGDYVSFDDIPQSALMRVKQWLVDEYDPATAHEPDFVEKLRDTKGIEGMILRLANGQSVKIKTQWYVDLHSQKDSVNVPKKLVTTILNGNHDDLYALFADDKPTIERIREFDSHVTKTLTNSFNAVRQFYARNRHLARKDYAIAGQKVLKPWEFGVAMIAYQKQTVEGVYESLVTAYLKRPELAIPEKYLNGV

SEQ ID NO: 3 - protein, 335 aa, Escherichia phage
MFKKYSSLENHYNSKFIEKLRTNGLTGGEWVAREKIHGTNFSLIIERDAVTCAKRTGPILPAEDFYGYEIVLKNYADSIKSIQDIMETSAAVSYQVFGEFAGTGIQKNVDYGDKDFYVFDIIVTTESGDVTYVDDYMMESFCKTFKFKMAPLLGRGKFEDLIKLPNDLDSVLPDYNFTVDNVGLAEANAHVWNAEAKGEVFTAEGYVLKPCYPLWLPNGNRVAIKCKNSKFSEKKKTDKPIKVAVVLSQDDLDLLQQFTDYVTVNRINNVISKIGEVSPKDFGKVMGLTVQDILEEAAREELELTDAENPVEVKKQLIECVKDTLRAVWIELVSK

SEQ ID NO: 4 - protein, 339 aa, Klebsiella phage
MFKKYSSLTNHYEGKFINGVIMNGLTGGVWVAREKIHGANFSFITDDGITVTPAKRTDVVKPAEDFYGCSAVVAKYSPGIRKMWETLKKTGTYDDLVIQVYGEFAGRGVQKDVDYGEKDFYVFDIRVNGEFLPDNLCSLISRSHGLKMAPLLGYGTFEEIKELPITFESVVNKANSGIGSDNTVYGEFVYPIMDVEEGNIAEGFVMKPVSPAFMPNGERVAIKCKTTKFTEKKAKKATRFNAPVSLSEKDKNQLDEFVCYLTENRVKNVLSKLDLASITAKDFGRIMGLTVQDAIEEISRNHGPFLEQFEDPAMAKKLFVTEAQNMIRPVWGKILNHEF

SEQ ID NO: 5 - protein, 335 aa, Vibrio phage
MFKKYSSLENHYNSKFIEKLYTNGLTTGVWVAREKIHGTNFSLIIERDNVTCAKRTGPILPAEDFYGYEIVLKKYDKAIKAVQEVMESISTSVPVSYQVFGEFAGGGIQKGVDYGEKDFYVFDIIINTESDDTYYMSDYEMQDFCNTFGFKMAPMLGRGTFDSLIMIPNDLDSVLAAYNSTASEDLVEANNCVFDANVIGDNTAEGYVLKPCFPKWLSNGTRVAIKCKNSKFSEKKKSDKPVKTQVPLTEIDKNLLDVLACYVTLNRVNNVISKIGTVTPKDFGKVMGLTVQDILEETSREGIVLTSSDNPNLVKKELVRMVQDVLRPAWIELVS

SEQ ID NO: 6 - protein, 335 aa, Vibrio phage
MSFVKYTSLENSYRQAFVDKCDMLGVREWVALEKIHGANFSFIVEFKPNEAQDGAEFTVTPAKRTSTIGANVMGDYDFYGCTSVVEAHTAKMEAISNWLWARGIINVGETIIVYGELAGKGVQKEVNYGDKDFWAYDILLPETGKFLDWDVVLEACEFAKVKTTHEIARGTLDELLRIDPLFRSFHTPADVDGDNVAEGFVVKQLRNEKRLHNGSRAILKVKNDKFKEKKNKAGKTPRAAVVLTEEQEKLHAAFSCYLTENRLRNVLSKLETVTQKQFGMISGLFIKDAKDEFERDELNETAIARDDWDVIKRSLTNIANEILRKNWLDILDGNF

SEQ ID NO: 7 - protein, 382 aa, Acidobacteriabacterium
MKQMYDNLKALTQKNDMFFSSIQTTPSNKPVEIFSYHIASYSDWLEPDAIECRGIMFDITDKENPVILSRPMEKFFNLGENPLALPEDVLPLVKTIEEKRDGSLISTYLDDGKLYTKSKGSLYSDQANDSNRFLMRSENKDFKQALKTLAELGYTANMEYTSPKNQIVLKYEKQELIVLNIRNTETGDYLTLDDLAELDAENPEHTIYTHIAERFVDYEEVDGMSDEDVERIRDMKGIEGYVLVGQNQRVKLKTDWYVNLHRLKDNINNNRRLVESVVESRTDDLRQLFEHDQGSIDKIKEFEQYVLSKIKSCLAEVRTVYERVKHLDRKHYAINAQRYVDYTPLFSVIMRQFDDYNEENVVENIKQIALKNVDDFIPMHYK

SEQ ID NO: 8 - protein, 334 aa, Salmonellaenterica
MFKKYSSLENHYNSKFIEKLYSLGLTGGEWVAREKIHGTNFSLIIERDKVTCAKRTGPILPAEDFFGYEIILKNYADSIKAVQDIMETSAVVTYQVFGEFAGPGIQKNVDYGDKDFYVFDIIVTTESGDVTYVDDYMMESFCNTFKFKMAPLLGRGKFEELIKLPNDLDSVVQDYNFTVDHAGLVDANKCVWNAEAKGEVFTAEGYVLKPCYPSWLPNRNRVAIKCKNSKFSEKKKSDKPIKTKVELSEADNKLMGILACYVTLNRVNNVISKIGEIGPKDFGKVMGLTVQDILEETSREGITLTQADNPSLIKKELVKMVQDVLRPAWIELVS

SEQ ID NO: 9 - protein, 334 aa, YersiniaphagevB_YepM_ZN18
MFKKYSSLENHYNSKFIEKLYSLGLTGGEWVAREKIHGTNFSLIIERDKVTCAKRTGPILPAEDFFGYEIILKNYEDSIKAVQDIMETSAVVSYQVFGEFAGPGIQKNVDYGDKDFYVFDIIVTTESGDVTYVDDYMMESFCNTFKFKMAPLLGRGKFEELIKLPNDLDSVVQDYNFTVDHAGLVDANKCVWKAEAKGEVFTAEGYVLKPCYPSWLHNGNRVAIKCKNSKFSEKKKSDKPIKAKVELSEADNKLVGILACYVTLNRVNNVISKIGEIGPKDFGKVMGLTVQDILEETSREGITLTQADNPSLVKKELVKMVQDVLRPAWIELVS

SEQ ID NO: 10 - protein, 334 aa, Shigella phage pSs-1
MFKKYSSLENHYNSKFIEKLYSLGLTGGEWVAREKIHGTNFSLIIERDKVTCAKRTGPILPAEDFFGYEIILKNYADSIKAVQDIMETSAVVSYQVFGEFAGPGIQKNVDYGDKDFYVFDIIVTTESGDVTYVDDYMMESFCNTFKFKMAPLLGRGKFEELIKLPNDLDSVVQDYNFTVDHAGLVDANKCVWNAEAKCEVFTAEGYVLKPCYPSWLPNRNRVAIKCKNSKFSEKKKSDKPIKAKVELSEADNKLVGILACYVTLNRVNNVISKIGEIGPKDFGKVMGLTVQDILEETSREGITLTQADSPSLVKKELVKMVQDVLRPAWIELVS

SEQ ID NO: 11 - protein, 347 aa, Buttiauxella phage vB_ButM_GuL6
MFVKYSSLTNHYEGKFINGVIMNGLTGGVWVAREKIHGANFSLITSDGEKVIPAKRSGEILPTEQFYGCEPVVARYAPAIRKLWDVINTAQQVSGIYVDSLVIQVYGEFAGRGVQKDVDYGEKDFYVFDIRVNGEFLHDNIVAVYAKSVGLKMAPLLAYGTFDEIRALPITFDSVVNLANSGAIPAHNGVEPEFKNFMTLKDGEGENIAEGFVMKPVHPAFMPNGERVAIKCKTTKFSEKKNKQANRFNAPAELSENDKAKLDVFTCYLTENRVKNVLSKIDSANLTAKDFGRVMGLTVQDALEEIERNYGPFIEQFENPTLAKKTFTNEASSLIRTNWGAILNNEF

SEQ ID NO: 12 - protein, 374 aa, Bacteriophage AR1
MQELFNNLMELCKDSQRKFFYSDDVSASGRTYRIFSYNYASYSDWLLPDALECRGIMFEMDGEKPVRIASRPMEKFFNLNENPFTMNIDLNDVDYILTKEDGSLVSTYLDGDEILFKSKGSIKSEQALMANGILMNINHHQLRDRLKELAEDGFTANFEFVAPTNRIVLAYQEMKIILLNIRENETGEYISYDDIYKDAALRPYLVERYEIDSPKWVEEAKNAENIEGYVAVMKDGSHFKIKSDWYVSLHSTKSSLDNPEKLFKTIIDGASDDLKAMYADDEYSYRKIEAFETTYLKYLDRALFLVLDCHNKHCGKDRKTYAMEAQGVAKGAGMDHLFGIIMSLYQGYDSQEKVMCEIEQNFLKNYKKFIPEGY

SEQ ID NO: 13 - protein, 381 aa, Vibrio phage
MTTQELYNHLMTLTDDAEGKFFFADHISPLGEKLRVFSYHIASYSDWLLPGALEARGIMFQLDEQDKMVRIVSRPMEKFFNLNENPFTMDLDLTTTVQLMDKADGSLISTYLTGENFALKSKTSIFSEQAVAANRYIKLPENRDLWEFCDDLTQAGCTVNMEWCAPNNRIVLEYPEAKLVILNIRDNETGDYVSFDDIPLPALMRVKKWLVDEYDPETAHADDFVEKLRATKGIEGMILRLANGQSVKIKTQWYVDLHSQKDSVNVPKKLVTTILNNNHDDLYALFADDKPTIDRIREFDSHVSKTVSASFHAVSQFYVKNRHMSRKDYAIAGQKTLKPWEFGVAMIAYQNQTVEGVYEALVGAYLKRPELLIPEKYLNEA

SEQ ID NO: 14 - protein, 381 aa, Vibrio phage phi-ST2; identical to SEQ ID NO: 2

SEQ ID NO: 15 - protein, 374 aa, Escherichia phage JN02
MEKLYYNLLSLCKSSSDRKFFYSDDVSPIGKKYRIFSYNFASYSDWLLPDALECRGIMFEMDGETPVRIASRPMEKFFNLNENPFTLSINLDDVKYLMTKEDGSLVSTYLDGGTVRFKSKGSIKSDQAVSATSILLDIDHKNLADRLLELCNDGFTANFEYVAPTNKIVLTYPEKRLILLNIRDNNTGEYIEYDDIYLDPVFRKYLVDRFEVPEGDWTSDVKSSTNIEGYVAVMKDGSHFKLKTDWYVALHTTRDSISSPEKLFLAIVNGASDDLKAMYADDEFSFKKVELFEKAYLDFLDRSFYICLDTYDKHKGKDRKTYAIEAQAVCKGAQTPWLFGIIMNLYQGGSKEQMMTALESVFIKNHKNFIPEGY

SEQ ID NO: 16 - protein, 339 aa, Klebsiella phage KP15
MFKKYSSLTNHYEGKFINGVIMNGLTGGVWVAREKIHGANFSFITDDGITVTPAKRTDVVKPAEDFYGCSAVVAKYSPGIRKMWETLKKTGTYDDLVIQVYGEFAGRGVQKDVDYGEKDFYVFDIRVNGEFLPDNLCSLISRSHGLKMAPLLGYGTFEEIKELPITFESVVNKANSGIGSDNTVYGEFVYPIMDVEEGNIAEGFVMKPVSPAFMPNGERVAIKCKTTKFTEKKAKKATRFNAPVSLSEKDKNQLDEFVCYLTENRVKNVLSKLDLASITAKDFGRIMGLTVQDAIEEISRNHGPFIEQFEDPAMAKKLFVTEAQNMIRPVWGKILNHEF

SEQ ID NO: 17 - protein, 334 aa, Vibrio phage JS98
MFKKYSSLENHYNSKFIEKLRTNGLTGGEWVAREKIHGTNFSLIIERDAVTCAKRTGPILPAEDFYGYEIVLKNYADSIKSVQHLIESINYQSYQIYGELAGPGIQKNVDYGDKDFYVFDIRVTKEDGTESVLTDTLMEAFCIIHKFKVAPCLATGSFEDLIKLPNDFDSVIPDYNFAVDNAGLTIANSTDFIPKVEGKVFTAEGFVLKPDIPTWLPNGNRVAIKCKNSKFSEKKKSDKPIKAAVVLSQDDMDLMWQFTDYVTVNRINNVISKIGEVSKKDFGKVMGLTVQDILEEAAREELELTDAENPVEVKKQLVECVKDTLRAVWIELVS

SEQ ID NO: 18 - protein, 438 aa, thermophilic bacteriophage RM378
MESMNVKYPVEYLIEHLNSFESPEVAVESLRKEGIMCKNRGDLYMFKYHLGCKFDKIYHLACRGAILRKTDSGWKVLSYPFDKFFNWGEELQPEIVNYYQTLRYASPLNEKRKAGFMFKLPMKLVEKLDGTCVVLYYDEGWKIHTLGSIDANGSIVKNGMVTTHMDKTYRELFWETFEKKYPPYLLYHLNSSYCYIFEMVHPDARVVVPYEEPNIILIGVRSVDPEKGYFEVGPSEEAVRIFNESGGKINLKLPAVLSQEQNYTLFRANRLQELFEEVTPLFKSLRDGYEVVYEGFVAVQEIAPRVYYRTKIKHPVYLELHRIKTTITPEKLADLFLENKLDDFVLTPDEQETVMKLKEIYTDMRNQLESSFDTIYKEISEQVSPEENPGEFRKRFALRLMDYHDKSWFFARLDGDEEKMQKSEKKLLTERIEKGLFK

SEQ ID NO: 19 - protein, 335 aa, Vibrio phage phi-ST2
MSFVKYTSLENSYRQAFVDKCDMLGVKEWVALEKIHGANFSFIVEFKPSTEEVPGEMSVTPAKRTSTIGANAMGDYDFYGCTSVVEAHIEKMQDISNWLFANDFIKNDETIIVYGELAGKGIQKEVNYGDKDFWAYDILCPETGEFLDWDVVLKACKFAGVKTTHEIARGTLDELLKIDPLFRSFHTPADVDSENVAEGFVVKQLKAEKRLHNGSRAILKVKNEKFKEKKNKQGKTPRAKVVLTEEQEKLHAAFSCYLTENRLRNVLSKIGKVEAKQFGMVSGLFVKDAKDEFERDERDEVAIPRDDWDVIKRSLVNVANEILRKNWLNIVDGTF

SEQ ID NO: 20-21 - skipped (2 entries)

SEQ ID NO: 22 - RNA, 10 nt, synthetic construct
  source 1..10: mol_type = other RNA
gactgcacta

SEQ ID NO: 23 - RNA, 11 nt, synthetic construct
  source 1..11: mol_type = other RNA
tctcactcact

SEQ ID NO: 24-27 - skipped (4 entries)

SEQ ID NO: 28 - RNA, 11 nt, synthetic construct
  source 1..11: mol_type = other RNA
tctcactcact

SEQ ID NO: 29 - skipped

SEQ ID NO: 30 - RNA, 12 nt, synthetic construct
  source 1..12: mol_type = other RNA
tcctgactatgt

SEQ ID NO: 31-32 - skipped (2 entries)

SEQ ID NO: 33 - RNA, 14 nt, synthetic construct
  source 1..14: mol_type = other RNA
aaattaactcaagt

SEQ ID NO: 34-35 - skipped (2 entries)

SEQ ID NO: 36 - RNA, 11 nt, synthetic construct
  source 1..11: mol_type = other RNA
gactgcactaa

SEQ ID NO: 37-41 - skipped (5 entries)

SEQ ID NO: 42 - RNA, 144 nt, synthetic construct
  source 1..144: mol_type = other RNA
agacctgcgactgcactatagtttaccatgtgcatccgagctcagcccttaagcatcagctgacttatcgtcgactaacagattattcgagctccatctgcttaatcttaggcttacctcgattctgcaatccattgtgctacc

SEQ ID NO: 43 - RNA, 144 nt, synthetic construct
  source 1..144: mol_type = other RNA
ggtagcacaatggattgcagaatcgaggtaagcctaagattaagcagatggagctcgaataatctgttagtcgacgataagtcagctgatgcttaagggctgagctcggatgcacatggtaaactatagtgcagtcgcaggtct